European Patent Application EP 4 403 634 A1, published July 24, 2024. Title: Antisense compound for modulating WFDC2 expression. Applicant: 1-2021-071500-1. Application KR 10-2022-0116229, filed September 15, 2022. The sequence listing filed with the application follows.

SEQUENCE LISTING (386 sequences)

SEQ ID NO: 1 - DNA, 11780 bp, synthetic construct
  source 1..11780: mol_type = other DNA
acacctgcaccccgcccgggcatagcaccatgcctgcttgtcgcctaggcccgctagccgccgccctcctcctcagcctgctgctgttcggcttcaccctagtctcaggtgagtggggcggggagaggcccggcgcctagaggggccgagccacgagcgccaggatggagccaggcggaggcgtagcctctggaggctggggaagtgggaattccgggggcggaagtggcggggacccttggagcctagggtgtggggtccaatgtgctggaggtggagagaccactgatggctgcaatttgggaggattctgtgctgaacgcggacactccgtggctgcagtgggctgggggtgggggctgctctgcctcgacctcggaagctccgagacgctcagctgtgcggcgtcccctagggctgagatctgagggccccgacgccaagggttagggagctctcgtactcccaggggtcagggactcctggtctggaagaaggagtctctgggggctgtaaggggactcctagggccagagactgagaattccttggggttaaggtttggagcaggaggtgggcatcctctggggctggcgctacgccccaccctcgactgtcccgggcctcccctcccaggcacaggagcagagaagactggcgtgtgccccgagctccaggctgaccagaactgcacgcaagagtgcgtctcggacagcgaatgcgccgacaacctcaagtgctgcagcgcgggctgtgccaccttctgctctctgcccaatggtaaccccacggcggccgagcgggaacggggcggggccgcgctgggctgggaggaggtgggagggcccgggttccgggaacaggggcgcccccggacccggggacccccgggaaagtcaaggcggttgaaaccagatccgtcagtcctctccctcgcacggcccaggggtagacaaaggcgtcgttgaaacgcagccaagggggggtccccacccctagctgggattcgagtctctggtgcatgacgggcttccgggcacgcacagccgggacattgttccccgcggcctggggacccggggccgcagtttccttctcgaaccggccgaagcctgccctgcgggaaagcccggagcctggggcgctcacctctcctcttggagtccctccctgggggcctcccccagccctggggaaagactgggagagcctggcctggcaagattttccccaattcctctgtccaggcggaaaggaactttacagatttaggaaaatgccccgctcatcttaaagatgtgtaagggagcatcggtgagaaaaaaatgttcttgcccaaggtcacaccgccatcccatggctgctggagtcatagtgagggttcagcttttgcctttcaggccaactggctgagtgattcgaagaaagtgaggaatcctccctggacactgtatcgcccttcgtcgtctttcagtcaatctcttccactctaaggattgagtgagcgcgagctggggactctctcaaaggtgcttgctggagctgcagtctccaccaggctatcagaacagggggtggcttaaacagcatggaatctcagctttccgttctccagaggaaaatgctgaggattagaggcagggataggacctggagagaaccaaggtactgtaatgatgttctttatccagaatacagcccctgtgacttttcctctctgttatttccttgaagatgccagcacaggctgggaaggtttgtaatacggtgacccaagacaccgatcagcagggaggtggtaagtggagggggactggcagcccaccaagggcagcttcaaggtcatgagtcccctcctctgggccagggagaggaggaccagaaggagagaggaagatttggagagaaagcaggcagcagccagatgagagaggtggaggagcaaaggagggagtctttgctgtttgatggatgaagaatttgttcccttatctcagatggacagactgaggcaggaagagggacaaggtcagatggcctcctgagccagggaggcagcctggaggtttgaatcctagttctgccattttctagttatgtgatcctgagcatgttgtttacctctctgagcctctgctctaagatgggaataattccaaactctataggattggcatgaggactaaatgaaataatgcatctaaagtgtctattagtgagaagatactccatacacagtggcttgttttgatcataaatggttccctatttatttccagggcagcccaatattacaggttcctactcctttcaagagaatgaatttctttgtattaggaagtcaagactgttggcaacttaacaacatttttttttgtatttatgctttaagttctggggtacacgtgcagaacgtgcaggtttgttacataggtatacatgtgccatggtggtttgcttcacccatcaacccgtcatctacattaggtgtttctcctaatgctatgcctcccctaattcccaaccccccgacaggccctggtgtgtgatgttcccctccctgtgtccatgtgttctcattgttcaactcctacttatgagtgagaacatgcggtatttggttttctgttcttgtgttagtttgctgagaatgatggtttccagcttcatccatgtctctgcaaaggacatgaactcatcatttgttatggctgcatagtattccatggtgtagacgtgccacatttcctttatccagtccatcactgatgggcatttgggttggttccaagtctttgctattgtgaacagtgctgcaataaacctatgtgtgcatgtgtcttgggcatttgcgttggttccaagtctttgctattgtgaacagtgctgcaataaacctatgtgtgcatgtgtctttattgtagaatgatttataatcctttgggtatatacccagtaatgggattgctgggtcaaatggtatttcttgttctagatccttgaggaatggccacactctcttccacaatggttgaactaatttacactcccacgaacagtgtaaaagcattcctatttctccacatcctctccagcatctgttgtttcctgactttttaaggatctccattctaactggtgtgagatgttatctcattgtggttttgatttgcatttctctaatgaccagtgatgatgagcatttttcatgtttgttggctgcataaatgtcttcttttgagaagcatctgttcatatccttcgcccacgttctaatggggtttttttctcgtaaatttgtttgagttcttgtagattctgtatattagccctttgtcagatggatagagtgcaaaaattttctcccattctgtaggctgcctgttcactctgatgatagtttcttttgctgtgcagaagctctgtagtttaattggatcccatttgtcaattttggcttttgttgccattgcttttggtgttttagtcatgaagtctttgcccatgcctatgtcctgaatggtattgcctaggttttcttctagggtttttatggttttaggtcttacatttaagtctttaatccatcttgagttaatttttgcataaggtgtaaggaaaggggtccagtttcagttttctgcatatggctagccagttttcccaacaccatttattaaatagggaatcctttccccattgcttgtttttgccatgtttgtcaaagatcaggtggctgtagatgtgtagtgttatttctgaggcctctgttctgttctgttggtctatatatctgttttggtaccagtaccatgctgttttggttactgtagccttgtagtatagcttgaagtcagttagcgtgatgcttccagctttgttctttttgcttaggattgtcttggctatgtgggcttttatttggttccatatgaaatttaaagtcgttttttctaattctgtgaagaaagtcagtgatagcttgatggggatagcattgaatctataaattactttgggcagtatagccattttcacgatattgattcttcttatccatgagcatggattgtttttccatttgtttgtatcctctcttatttcgttgagcagtggtttgtagttctccttgaagaggtccttcacctcccttgtaagttgtattcctaggtattttattctctttgtagcaattgtgaatgggaattcactcatgatttggctctctgtctattattggtgtataggaatacttgtgatttttgtacattgatttgtatcctgagactttactgcagtttcttatcagcttaaggagattttgggctgagataatggggttttctaaatatacaatcatttcatctgcaaacagggacaatttgacttcctcttttcctaattgaataccctttatttctttctcttgactgattgccctggccagaatttctaatgctatgttgaataggggtggtgagagagagcatgcttgtcttgtgccggttttcaaagggaatgcttccagcttttgcccattcagtatgatattggctgtgggtttgtcataaatagctcttgttactttgagataccttccatcaatacctagtttattgagtgttttagcatgaagggtgttgaattttatcaaaggccttttctgcatctattgagataatcatgtggtttttgtcattgattttgcttatgtgatggattacgtttattgatttgtgtatgttgaaccagccttgcatcccagggacaaagccaacttgatcatggtggataagctttttgatgtgctgctggatttggtttgccagcattttattaaggattttcgcactgatgttcatcagggatattaacctgaaatttttttgttattgtgtctctgccaggttttagtatcaggatgatgctggcctcataaaatgaattagggaggaggctctctttttctattgtttggaatagtttcagaaggaatggtaccagcaactcctctttgtacctctggtggaattcggctgtgaatctgtctggtcccagactttttttggttggtaggctattaattactgcctcaattttggaacttgttattggtcgattcagggattcgacttcttcctggtttagacttgggagggtgtatgtgtccaggaatttatccatttcttctaggttttctagtttatttgcgtagaggtgtttatagtattctctgatggtagattgtatttctgtgggatcagtggtgatatcccctttgtcattttttattgtgtctatttgattcttctctcttttctttattagtatggctagcagtcagactattttgttgatgtttttcaaaaacccagcttgtgaattcattgattttttttgaagggtttttcatgtctctatctcctttagttctctctgatcttagttatttcttgtcttctgctagcttttgaatttgtttgttcttgcttttctagttcttttaattgtgatgttagggtgtcaattttggatctttcctgctttcccttgtgggcatttagtgctataaatttccttctaagcactgctttagctgtgtctcagagattctggtatgttatgtctttgttctcattggtttcaaagaacttatttatttctgccttgattttgttatttacctagtagtcattcaggagcaggttgttcagtttccatgtaaggttatgcggtcttgagtgagtttcttaatcctgaattctaatttgatggcactgtggtctgagagactgttaggatttccgttcttttgcatttgctaattagtgttttacttccaattatgtggtcagttttagaataagtgtgatgtggtgctgaggagaatgtatattctgttgatttggggtggagagttctgtagatgtctattaggtctgcttggtccagagctgagttcaagtcttggatatctttgttaattttccgtctcattgatctgtctaatattgacagtgggggttaaagtttcccactattattatgtcggagtctaagtctctttgtaggtctctaagaacttgctttatgaatcagggtgctcctgtattaggtgcatatatatttagcataattagctcttcttgttgcattgatccctttaccattgtgtaatgcccttctttgtctcttttgatctttgttggtttaaagtctgttttatcagagaatagaattgcaacccctgatttttttttgctttccatttgcttggtaaatattcctctatccctttattttgagcctatgtgtctttgcacttgagatgggtctcctgaatacagcacaccaatgggtcttgactctttatccaatttgccagtctttgtcttttaactggggcatttagcctgtttacatttaaggttaatattgttatgtgtgagtttgatcctgtcattatgatgctagctggttattttgtctattagttgatgcagtttcttcatagtgtcgatggtctttacaatttggtatgtttttgcagttgctgattccagttgttcctttctatgtttagtgctcctttcaggagaccttgtaaggcaggcctgttgatgagaaaaatccctcagcatttgtttgtctataaaggattttatttctccttcatgtatgaagcttactttggctggatatgaaattctgggttgaaaattctttaagaatattgaatattggcccccactgtcttctggtttgcagggtttctgcagagagatctgcagttagtctgaagggcctcccatagtgggtaacccaacctttctctctgggtgcccttaacatttttttcttcatttcaaccttggtgaatctgatgattatgtgtcttggggttattcttctcaaggagtatctttgaggtgttctctgtatttcctgaatttgaatgttggcctttcttgctaggttggggaagttctcctgtataatatcctgaacagtgttttccaacttggttccattctccccatcactttcaggtacatcaatcaaacataggtttggtcttttcacatagtcccatattttttggaggctttgttcattcattccttttcattattttttctctaatctcatcttcattctttatttcattaaattgatcttcaatctctgatatccttcttctgcttgatcaattcggctattgatacttgtataggcttcatgacgttctcgtgctgtgtttttcagctccatcaggtcatttatgttcttctctaaactggttaatctagttagcaattcctataaccttttttcaaggttcttacctttcttgcattggggttagaacatgctcctttagcttggaggagtttgttattacccaccttctgaagcctacttctgtcaatttgtcaaactcattctccgtccagttttgttcccttgctggcgaggaattgtgatcctttggagaagaggtgttctggtttttggaattttcagcctttttgtgctggtttctccccatcttcgtggatttatctacctttggtctttgatgttgatgatctttggatgggccttctgagtggacgtcctttttgttgatgttgatgctattcctttctgttagttttccttctaacaatcaggcccctcagctgcaggtctgttggcgtttgctggaggtccactccagaccctgtttgcctggctatcaccagcagaggctgcagaacagcaaagattgctgcctgttccttcctctagaagctttgtcccagaggggcacccgccagatgccagccagagctctcctgtatgaggtgtctgtcagcccctgctggaaggtgtctcccagtcaggagacacggaaatcagggactcacttgaggaggcagtctgacccttagcagagctcaaatgctgtgctgggagatctgctgctctcttcagaaccggcaggcaggctgaagccacatccacagctgccccttcccccaggtgctctgtcccagggagatgggagttttacctataagcccctgactagggctgctgcctttttttcagagatgccctgcccagagaggaggaatctagagaggcagtctggctacagcggctttgccgagctgtgttgggctctgcccagtttgaacttcctggtggctttgtttactctgtgaggggaaaactgcctactcaagcctcagtaatggtggacgcccctccccctaccaagcttgagagttccaggtcaacttcagactgctgtgctggcagtgagaatttcaagccagtggatgttagcttgctgggctccatgggggtgggatccgctgagctagaccacttgtctccctagcttcagccccctttccaggggcgtgaatggttctgtctcactggcattccaggcaccactggggtatgaaaaaaaaatcctgcagctagctcagtgtctgcccaaatggccacctagttttgtgcttgaaacccagggccctggtggtgtaggcacccaaaggaatctcttggtctgtgggttgtgaagaccgtgggaaaagtgtagtatctgctccagagtgcactattcctcacggcacagtccctcatggcttcccttggctaggggagggagttccctgacctcttgtgcttcccaggtgagatgatgccctaccctacttctgctcgccctccgtgggctgcacccactgtctaaccagtcccaatgagatgagccacgtacctcatttgaaaatgcagaaatcacctgccttctgcattgattcactgggagctgcagactggagctgttactattcggccatcttgaaagctgaacctaaatcttttttttttttgagatggagtctcgctctgtcgcccaggctggagtgcagtggcatgatctcagctcactacaacctctgtctcccaggtgcaagcgattctcctgcctcagcctcccaagtagctgggattaccggtgcatgccaccacgcccagttaacttttttgtatttttagtagagcggggggtctcgagtcctgacctccgatgatcccacccgcctgagcctcccaaagtgtgggattacaggcatgagccactgcacccggtgatctgtcagccactttccttgtcctctacagctaatcacccagttctgtgcctgtgttttacacacaaaaacctgcacatatttatagcagctttatttataattgccaaaagttggaagcaaccatgatgtacctcagttgatgaatggatttggctgggcctggctcccctctatctaacctgggaagtggagtgtgattgtgtgtgtgtttgttagtggaaggacgtgtggtttctctctgcatggatgaatgagtgtatttggagggtcatggtgctgagagactgcaactgggattcggtctgtgggtatgagtgaagattataagtgtgtaacccctcacatgtgtactgtactttacactttaagtggcagcatagtgcttaaccatggcagcagcagttaacacatagactctgcagctagatttcttggggttcaaattctgcctcaattctgtgtgaccttaggcaaattacttaacttctcagtgcctcagtttcctcacttgtaacacaaggaaatattaacagatccctccccttcttttaggattattgtgagaattagaagagttaatatatgttaggggcttgatacctggcatgtaataagagctaattaagtgttcactgttataatttctcataactacagagtagtttgatatttcagggagaaataatatatgtttgtttcccactgctttcacaacaaccctatgttgtaattagcactgttccactggcacctaaagacacggaggctctgggagatttctggccctaggccacgaaggcccacttgggactcaagctgaggtcctgtgattccatttgggagcaggaggagggatttgcaggtgatcttcctgggcctcctgagagcagctcaggtgcccaagatggactcaggcaggcagctctgctgtatgtgaagcccagtgaggggcagtgggggggccatgctgcaggtacaagttaatctccctgtatcgcctctgcccacttacccttactcctttttctacccagataaggagggttcctgcccccaggtgaacattaactttccccagctcggcctctgtcgggaccagtgccaggtggacagccagtgtcctggccagatgaaatgctgccgcaatggctgtgggaaggtgtcctgtgtcactcccaatttctgaggtaagtgaacgggaaagagaaagtgcattgatggccaggtgttgtgggaaacaggagaaaacgtcacccaggcggaggtgaagggaggttagttgcagggacagttgggaaaggtataccagtggggtgaccctcagcctgttctaaaagaagagtgaaaggtgggtagtctgatgagctgcattggggaggctgtctcaggcagagggaacagaataagcaagagcttggctgggtgtggtggctcatgcctataatcccagcactttgggaggctgaggtgtgcggatcacctgaggtcgggagttcaagaccagcctgaccaacatggagaaaccccgtctctactaaaaataccaaaaaaaaaaaaaaaaatttaatgggtgtggtggcgggtgccacccacccgctactcaggaggctgaggcaggagaattgcttgaacctgggagacagaggttgtggtgagctgagatcacgccattgcactccagcctgggcaacaagagcgaaactccatctcaaattaaaaacaaacaaacaaaaaacagcttggtggtacccttgggttgaaatctcgtggttgtcatgtgctacttttaacaatttctcagcaaagtaacctgaagataactgatagaatccaatagtgcagagatgagcaattgaaatctagagagggggtgtgctcttggtgcccgagagggaactatggtttctctaaactaagctatggtctccctggagccagggctctcagatgccaactgcatggataggctttgcagtcaagaagaccttggttcaaatgttagctctgacacttacctaaccttctcacctccctgagtcacagttatctcgcttataaaatgtagctaaataagatctaattgatcagataatcccattttaacctaaagaagaaggcatggcagaacttcctaatagtagaaggattcttggggagagaaatggccatgacccctcaggaaggccacagtggacatctgggaccacagtatacccaggtgcctgctagggatggtctgaccacagtatacccaggtacctgctagggatggtctgaaggagaagagtatgtctagaacctgtagaaaatgcaagcagagcccccagaaggtgaggctttgctgtgtgggtgtgtgggatggggtggggtcaaggagctggtctaggatttaagctgcaggtactcctgcctagtctaatggatattgttgttgatggtattgttataattttcttcctccagctccagccaccaccaggctgagcagtgaggagagaaagtttctgcctggccctgcatctggttccagcccacctgccctcccctttttcgggactctgtattccctcttgggctgaccacagcttctccctttcccaaccaataaagtaaccactttcagca

SEQ ID NO: 2 - DNA, 567 bp, synthetic construct
  source 1..567: mol_type = other DNA
acacctgcaccccgcccgggcatagcaccatgcctgcttgtcgcctaggcccgctagccgccgccctcctcctcagcctgctgctgttcggcttcaccctagtctcaggcacaggagcagagaagactggcgtgtgccccgagctccaggctgaccagaactgcacgcaagagtgcgtctcggacagcgaatgcgccgacaacctcaagtgctgcagcgcgggctgtgccaccttctgctctctgcccaatgataaggagggttcctgcccccaggtgaacattaactttccccagctcggcctctgtcgggaccagtgccaggtggacagccagtgtcctggccagatgaaatgctgccgcaatggctgtgggaaggtgtcctgtgtcactcccaatttctgagctccagccaccaccaggctgagcagtgaggagagaaagtttctgcctggccctgcatctggttccagcccacctgccctcccctttttcgggactctgtattccctcttgggctgaccacagcttctccctttcccaaccaataaagtaaccactttcagca

SEQ ID NO: 3 - DNA, 20 bp, synthetic construct
  source 1..20: mol_type = other DNA
tgctctctgcccaatgataa

SEQ ID NO: 4 - DNA, 20 bp, synthetic construct
  source 1..20: mol_type = other DNA
ttgggagtgacacaggacac

SEQ ID NO: 5 - DNA, 20 bp, synthetic construct
  source 1..20: mol_type = other DNA
ctgacttcaacagcgacacc

SEQ ID NO: 6 - DNA, 20 bp, synthetic construct
  source 1..20: mol_type = other DNA
ggtggtccaggggtcttact

SEQ ID NO: 7 - DNA, 20 bp, synthetic construct
  source 1..20: mol_type = other DNA
gcgacaagcaggcatggtgc

SEQ ID NO: 8 - DNA, 20 bp, synthetic construct
  source 1..20: mol_type = other DNA
aggcgacaagcaggcatggt

SEQ ID NO: 9 - DNA, 20 bp, synthetic construct
  source 1..20: mol_type = other DNA
ccattgcggcagcatttcat

SEQ ID NO: 10 - DNA, 20 bp, synthetic construct
  source 1..20: mol_type = other DNA
ccccactcacctgagactag

SEQ ID NO: 11 - DNA, 20 bp, synthetic construct
  source 1..20: mol_type = other DNA
aattcccacttccccagcct

SEQ ID NO: 12 - DNA, 20 bp, synthetic construct
  source 1..20: mol_type = other DNA
ggaattcccacttccccagc

SEQ ID NO: 13 - DNA, 20 bp, synthetic construct
  source 1..20: mol_type = other DNA
ccacctccagcacattggac

SEQ ID NO: 14 - DNA, 20 bp, synthetic construct
  source 1..20: mol_type = other DNA
tccacctccagcacattgga

SEQ ID NO: 15 - DNA, 20 bp, synthetic construct
  source 1..20: mol_type = other DNA
tctccacctccagcacattg

SEQ ID NO: 16 - DNA, 20 bp, synthetic construct
  source 1..20: mol_type = other DNA
ctctccacctccagcacatt

SEQ ID NO: 17 - DNA, 20 bp, synthetic construct
  source 1..20: mol_type = other DNA
agtggtctctccacctccag

SEQ ID NO: 18 - DNA, 20 bp, synthetic construct
  source 1..20: mol_type = other DNA
gcagccatcagtggtctctc

SEQ ID NO: 19 - DNA, 20 bp, synthetic construct
  source 1..20: mol_type = other DNA
aaattgcagccatcagtggt

SEQ ID NO: 20 - DNA, 20 bp, synthetic construct
  source 1..20: mol_type = other DNA
ccaaattgcagccatcagtg

SEQ ID NO: 21 - DNA, 20 bp, synthetic construct
  source 1..20: mol_type = other DNA
agaatcctcccaaattgcag

SEQ ID NO: 22 - DNA, 20 bp, synthetic construct
  source 1..20: mol_type = other DNA
cacagaatcctcccaaattg

SEQ ID NO: 23 - DNA, 20 bp, synthetic construct
  source 1..20: mol_type = other DNA
tccgcgttcagcacagaatc

SEQ ID NO: 24 - DNA, 20 bp, synthetic construct
  source 1..20: mol_type = other DNA
agtgtccgcgttcagcacag

SEQ ID NO: 25 - DNA, 20 bp, synthetic construct
  source 1..20: mol_type = other DNA
ccctcagatctcagccctag

SEQ ID NO: 26 - DNA, 20 bp, synthetic construct
  source 1..20: mol_type = other DNA
cgagagctccctaacccttg

SEQ ID NO: 27 - DNA, 20 bp, synthetic construct
  source 1..20: mol_type = other DNA
acgagagctccctaaccctt

SEQ ID NO: 28 - DNA, 20 bp, synthetic construct
  source 1..20: mol_type = other DNA
tacgagagctccctaaccct

SEQ ID NO: 29 - DNA, 20 bp, synthetic construct
  source 1..20: mol_type = other DNA
gagtacgagagctccctaac

SEQ ID NO: 30 - DNA, 20 bp, synthetic construct
  source 1..20: mol_type = other DNA
tccagaccaggagtccctga

SEQ ID NO: 31 - DNA, 20 bp, synthetic construct
  source 1..20: mol_type = other DNA
ttccagaccaggagtccctg

SEQ ID NO: 32 - DNA, 20 bp, synthetic construct
  source 1..20: mol_type = other DNA
cttcttccagaccaggagtc

SEQ ID NO: 33 - DNA, 20 bp, synthetic construct
  source 1..20: mol_type = other DNA
gactccttcttccagaccag

SEQ ID NO: 34 - DNA, 20 bp, synthetic construct
  source 1..20: mol_type = other DNA
agagactccttcttccagac

SEQ ID NO: 35 - DNA, 20 bp, synthetic construct
  source 1..20: mol_type = other DNA
cccagagactccttcttcca

SEQ ID NO: 36 - DNA, 20 bp, synthetic construct
  source 1..20: mol_type = other DNA
cccagagactccttcttcca

SEQ ID NO: 37 - DNA, 18 bp, synthetic construct
  source 1..18: mol_type = other DNA
acactggctgtccacctg

SEQ ID NO: 38 - DNA, 20 bp, synthetic construct
  source 1..20: mol_type = other DNA
tttcatctggccaggacact

SEQ ID NO: 39 - DNA, 18 bp, synthetic construct
  source 1..18: mol_type = other DNA
gcagcacttgaggttgtc

SEQ ID NO: 40 - DNA, 18 bp, synthetic construct
  source 1..18: mol_type = other DNA
caggcatggtgctatgcc

SEQ ID NO: 41 - DNA, 20 bp, synthetic construct
  source 1..20: mol_type = other DNA
gcgttcagcacagaatcctc

SEQ ID NO: 42 - DNA, 20 bp, synthetic construct
  source 1..20: mol_type = other DNA
agctgagcgtctcggagctt

SEQ ID NO: 43 - DNA, 20 bp, synthetic construct
  source 1..20: mol_type = other DNA
tccttcttccagaccaggag

SEQ ID NO: 44 - DNA, 20 bp, synthetic construct
  source 1..20: mol_type = other DNA
agactccttcttccagacca

SEQ ID NO: 45 - DNA, 20 bp, synthetic construct
  source 1..20: mol_type = other DNA
ccctaggagtccccttacag

SEQ ID NO: 46 - DNA, 20 bp, synthetic construct
  source 1..20: mol_type = other DNA
agtctctggccctaggagtc

SEQ ID NO: 47 - DNA, 20 bp, synthetic construct
  source 1..20: mol_type = other DNA
tcagtctctggccctaggag

SEQ ID NO: 48 - DNA, 20 bp, synthetic construct
  source 1..20: mol_type = other DNA
ttctcagtctctggccctag

SEQ ID NO: 49 - DNA, 20 bp, synthetic construct
  source 1..20: mol_type = other DNA
attctcagtctctggcccta

SEQ ID NO: 50 - DNA, 20 bp, synthetic construct
  source 1..20: mol_type = other DNA
caaggaattctcagtctctg

SEQ ID NO: 51 - DNA, 20 bp, synthetic construct
  source 1..20: mol_type = other DNA
cccaaggaattctcagtctc

SEQ ID NO: 52 - DNA, 20 bp, synthetic construct
  source 1..20: mol_type = other DNA
accccaaggaattctcagtc

SEQ ID NO: 53 - DNA, 20 bp, synthetic construct
  source 1..20: mol_type = other DNA
taaccccaaggaattctcag

SEQ ID NO: 54 - DNA, 20 bp, synthetic construct
  source 1..20: mol_type = other DNA
ttaaccccaaggaattctca

SEQ ID NO: 55 - DNA, 20 bp, synthetic construct
  source 1..20: mol_type = other DNA
ccttaaccccaaggaattct

SEQ ID NO: 56 - DNA, 20 bp, synthetic construct
  source 1..20: mol_type = other DNA
accttaaccccaaggaattc

SEQ ID NO: 57 - DNA, 20 bp, synthetic construct
  source 1..20: mol_type = other DNA
aaccttaaccccaaggaatt

SEQ ID NO: 58 - DNA, 20 bp, synthetic construct
  source 1..20: mol_type = other DNA
ccaaaccttaaccccaagga

SEQ ID NO: 59 - DNA, 20 bp, synthetic construct
  source 1..20: mol_type = other DNA
ctccaaaccttaaccccaag

SEQ ID NO: 60 - DNA, 20 bp, synthetic construct
  source 1..20: mol_type = other DNA
ctcctgctccaaaccttaac

SEQ ID NO: 61 - DNA, 20 bp, synthetic construct
  source 1..20: mol_type = other DNA
tgcccacctcctgctccaaa

SEQ ID NO: 62 - DNA, 20 bp, synthetic construct
  source 1..20: mol_type = other DNA
atgcccacctcctgctccaa

SEQ ID NO: 63 - DNA, 20 bp, synthetic construct
  source 1..20: mol_type = other DNA
attgcggcagcatttcatct

SEQ ID NO: 64 - DNA, 20 bp, synthetic construct
  source 1..20: mol_type = other DNA
cattgcggcagcatttcatc

SEQ ID NO: 65 - DNA, 20 bp, synthetic construct
  source 1..20: mol_type = other DNA
gccattgcggcagcatttca

SEQ ID NO: 66 - DNA, 20 bp, synthetic construct
  source 1..20: mol_type = other DNA
agccattgcggcagcatttc

SEQ ID NO: 67 - DNA, 20 bp, synthetic construct
  source 1..20: mol_type = other DNA
cagccattgcggcagcattt

SEQ ID NO: 68 - DNA, 20 bp, synthetic construct
  source 1..20: mol_type = other DNA
aggacactggctgtccacct

SEQ ID NO: 69 - DNA, 20 bp, synthetic construct
  source 1..20: mol_type = other DNA
cttcccacagccattgcggc

SEQ ID NO: 70 - DNA, 20 bp, synthetic construct
  source 1..20: mol_type = other DNA
ggacactggctgtccacctg

SEQ ID NO: 71 - DNA, 20 bp, synthetic construct
  source 1..20: mol_type = other DNA
caggacactggctgtccacc

SEQ ID NO: 72 - DNA, 20 bp, synthetic construct
  source 1..20: mol_type = other DNA
acactggctgtccacctggc

SEQ ID NO: 73 - DNA, 20 bp, synthetic construct
  source 1..20: mol_type = other DNA
gacactggctgtccacctgg

SEQ ID NO: 74 - DNA, 20 bp, synthetic construct
  source 1..20: mol_type = other DNA
agcaggcatggtgctatgcc

SEQ ID NO: 75 - DNA, 20 bp, synthetic construct
  source 1..20: mol_type = other DNA
caggcatggtgctatgcccg

SEQ ID NO: 76 - DNA, 20 bp, synthetic construct
  source 1..20: mol_type = other DNA
tcctgtgcctgagactaggg

SEQ ID NO: 77 - DNA, 20 bp, synthetic construct
  source 1..20: mol_type = other DNA
gctcctgtgcctgagactag

SEQ ID NO: 78 - DNA, 20 bp, synthetic construct
  source 1..20: mol_type = other DNA
gtcttctctgctcctgtgcc

SEQ ID NO: 79 - DNA, 20 bp, synthetic construct
  source 1..20: mol_type = other DNA
cagtcttctctgctcctgtg

SEQ ID NO: 80 - DNA, 20 bp, synthetic construct
  source 1..20: mol_type = other DNA
acaccttcccacagccattg

SEQ ID NO: 81 - DNA, 20 bp, synthetic construct
  source 1..20: mol_type = other DNA
gacaccttcccacagccatt

SEQ ID NO: 82 - DNA, 20 bp, synthetic construct
  source 1..20: mol_type = other DNA
tcactgctcagcctggtggt

SEQ ID NO: 83 - DNA, 20 bp, synthetic construct
  source 1..20: mol_type = other DNA
ctctcctcactgctcagcct

SEQ ID NO: 84 - DNA, 20 bp, synthetic construct
  source 1..20: mol_type = other DNA
tttctctcctcactgctcag

SEQ ID NO: 85 - DNA, 20 bp, synthetic construct
  source 1..20: mol_type = other DNA
gaaactttctctcctcactg

SEQ ID NO: 86 - DNA, 20 bp, synthetic construct
  source 1..20: mol_type = other DNA
ggcagaaactttctctcctc

SEQ ID NO: 87 - DNA, 20 bp, synthetic construct
  source 1..20: mol_type = other DNA
agggccaggcagaaactttc

SEQ ID NO: 88 - DNA, 20 bp, synthetic construct
  source 1..20: mol_type = other DNA
atgcagggccaggcagaaac

SEQ ID NO: 89 - DNA, 20 bp, synthetic construct
  source 1..20: mol_type = other DNA
tgggctggaaccagatgcag

SEQ ID NO: 90 - DNA, 20 bp, synthetic construct
  source 1..20: mol_type = other DNA
gggaatacagagtcccgaaa

SEQ ID NO: 91 - DNA, 20 bp, synthetic construct
  source 1..20: mol_type = other DNA
ccaagagggaatacagagtc

SEQ ID NO: 92 - DNA, 20 bp, synthetic construct
  source 1..20: mol_type = other DNA
agctgtggtcagcccaagag

SEQ ID NO: 93 - DNA, 20 bp, synthetic construct
  source 1..20: mol_type = other DNA
tactttattggttgggaaag

SEQ ID NO: 94 - DNA, 20 bp, synthetic construct
  source 1..20: mol_type = other DNA
gtggttactttattggttgg

SEQ ID NO: 95 - DNA, 20 bp, synthetic construct
  source 1..20: mol_type = other DNA
tgaaagtggttactttattg

SEQ ID NO: 96 - DNA, 20 bp, synthetic construct
  source 1..20: mol_type = other DNA
tgctgaaagtggttacttta

SEQ ID NO: 97 - DNA, 20 bp, synthetic construct
  source 1..20: mol_type = other DNA
tgtgcctgagactagggtga

SEQ ID NO: 98 - DNA, 20 bp, synthetic construct
  source 1..20: mol_type = other DNA
gcacacgccagtcttctctg

SEQ ID NO: 99 - DNA, 20 bp, synthetic construct
  source 1..20: mol_type = other DNA
ttctggtcagcctggagctc

SEQ ID NO: 100 - DNA, 20 bp, synthetic construct
  source 1..20: mol_type = other DNA
ttgcgtgcagttctggtcag

SEQ ID NO: 101 - DNA, 20 bp, synthetic construct
  source 1..20: mol_type = other DNA
acttgaggttgtcggcgcat

SEQ ID NO: 102 - DNA, 20 bp, synthetic construct
  source 1..20: mol_type = other DNA
gctgcagcacttgaggttgt

SEQ ID NO: 103 - DNA, 20 bp, synthetic construct
  source 1..20: mol_type = other DNA
tatcattgggcagagagcag

SEQ ID NO: 104 - DNA, 20 bp, synthetic construct
  source 1..20: mol_type = other DNA
gaaagttaatgttcacctgg

SEQ ID NO: 105 - DNA, 20 bp, synthetic construct
  source 1..20: mol_type = other DNA
atttcatctggccaggacac

SEQ ID NO: 106 - DNA, 20 bp, synthetic construct
  source 1..20: mol_type = other DNA
agaaattgggagtgacacag

SEQ ID NO: 107 - DNA, 20 bp, synthetic construct
  source 1..20: mol_type = other DNA
tccttatcattgggcagaga

SEQ ID NO: 108 - DNA, 20 bp, synthetic construct
  source 1..20: mol_type = other DNA
aggaaccctccttatcattg

SEQ ID NO: 109 - DNA, 20 bp, synthetic construct
  source 1..20: mol_type = other DNA
tggccatcaatgcactttct

SEQ ID NO: 110 - DNA, 20 bp, synthetic construct
  source 1..20: mol_type = other DNA
ttttctcctgtttcccacaa

SEQ ID NO: 111 - DNA, 20 bp, synthetic construct
  source 1..20: mol_type = other DNA
tatacctttcccaactgtcc

SEQ ID NO: 112 - DNA, 20 bp, synthetic construct
  source 1..20: mol_type = other DNA
cactggtatacctttcccaa

SEQ ID NO: 113 - DNA, 20 bp, synthetic construct
  source 1..20: mol_type = other DNA
cttcttttagaacaggctga

SEQ ID NO: 114 - DNA, 20 bp, synthetic construct
  source 1..20: mol_type = other DNA
cctttcactcttcttttaga

SEQ ID NO: 115 - DNA, 20 bp, synthetic construct
  source 1..20: mol_type = other DNA
actacccacctttcactctt

SEQ ID NO: 116 - DNA, 20 bp, synthetic construct
  source 1..20: mol_type = other DNA
aatgcagctcatcagactac

SEQ ID NO: 117 - DNA, 20 bp, synthetic construct
  source 1..20: mol_type = other DNA
ttgcttattctgttccctct

SEQ ID NO: 118 - DNA, 20 bp, synthetic construct
  source 1..20: mol_type = other DNA
caagctcttgcttattctgt

SEQ ID NO: 119 - DNA, 20 bp, synthetic construct
  source 1..20: mol_type = other DNA
tgctgggattataggcatga

SEQ ID NO: 120 - DNA, 20 bp, synthetic construct
  source 1..20: mol_type = other DNA
tcccaaagtgctgggattat

SEQ ID NO: 121 - DNA, 20 bp, synthetic construct
  source 1..20: mol_type = other DNA
ggtatttttagtagagacgg

SEQ ID NO: 122 - DNA, 20 bp, synthetic construct
  source 1..20: mol_type = other DNA
caggttcaagcaattctcct

SEQ ID NO: 123 - DNA, 20 bp, synthetic construct
  source 1..20: mol_type = other DNA
ttgagatggagtttcgctct

SEQ ID NO: 124 - DNA, 20 bp, synthetic construct
  source 1..20: mol_type = other DNA
aaagtagcacatgacaacca

SEQ ID NO: 125 - DNA, 20 bp, synthetic construct
  source 1..20: mol_type = other DNA
gaaattgttaaaagtagcac

SEQ ID NO: 126 - DNA, 20 bp, synthetic construct
  source 1..20: mol_type = other DNA
tactttgctgagaaattgtt

SEQ ID NO: 127 - DNA, 20 bp, synthetic construct
  source 1..20: mol_type = other DNA
ttatcttcaggttactttgc

SEQ ID NO: 128 - DNA, 20 bp, synthetic construct
  source 1..20: mol_type = other DNA
attctatcagttatcttcag

SEQ ID NO: 129 - DNA, 20 bp, synthetic construct
  source 1..20: mol_type = other DNA
tgcactattggattctatca

SEQ ID NO: 130 - DNA, 20 bp, synthetic construct
  source 1..20: mol_type = other DNA
aattgctcatctctgcacta

SEQ ID NO: 131 - DNA, 20 bp, synthetic construct
  source 1..20: mol_type = other DNA
ctagatttcaattgctcatc

SEQ ID NO: 132 - DNA, 20 bp, synthetic construct
  source 1..20: mol_type = other DNA
accccctctctagatttcaa

SEQ ID NO: 133 - DNA, 20 bp, synthetic construct
  source 1..20: mol_type = other DNA
ttagagaaaccatagttccc

SEQ ID NO: 134 - DNA, 20 bp, synthetic construct
  source 1..20: mol_type = other DNA
ccatagcttagtttagagaa

SEQ ID NO: 135 - DNA, 20 bp, synthetic construct
  source 1..20: mol_type = other DNA
caaagcctatccatgcagtt

SEQ ID NO: 136 - DNA, 20 bp, synthetic construct
  source 1..20: mol_type = other DNA
ttcttgactgcaaagcctat

SEQ ID NO: 137 - DNA, 20 bp, synthetic construct
  source 1..20: mol_type = other DNA
aaccaaggtcttcttgactg

SEQ ID NO: 138 - DNA, 20 bp, synthetic construct
  source 1..20: mol_type = other DNA
aacatttgaaccaaggtctt

SEQ ID NO: 139 - DNA, 20 bp, synthetic construct
  source 1..20: mol_type = other DNA
tgtcagagctaacatttgaa

SEQ ID NO: 140 - DNA, 20 bp, synthetic construct
  source 1..20: mol_type = other DNA
aggttaggtaagtgtcagag

SEQ ID NO: 141 - DNA, 20 bp, synthetic construct
  source 1..20: mol_type = other DNA
gaggtgagaaggttaggtaa

SEQ ID NO: 142 - DNA, 20 bp, synthetic construct
  source 1..20: mol_type = other DNA
agcgagataactgtgactca

SEQ ID NO: 143 - DNA, 20 bp, synthetic construct
  source 1..20: mol_type = other DNA
gctacattttataagcgaga

SEQ ID NO: 144 - DNA, 20 bp, synthetic construct
  source 1..20: mol_type = other DNA
ggattatctgatcaattaga

SEQ ID NO: 145 - DNA, 20 bp, synthetic construct
  source 1..20: mol_type = other DNA
taaaatgggattatctgatc

SEQ ID NO: 146 - DNA, 20 bp, synthetic construct
  source 1..20: mol_type = other DNA
ttctttaggttaaaatggga

SEQ ID NO: 147 - DNA, 20 bp, synthetic construct
  source 1..20: mol_type = other DNA
ccatgccttcttctttaggt

SEQ ID NO: 148 - DNA, 20 bp, synthetic construct
  source 1..20: mol_type = other DNA
tattaggaagttctgccatg

SEQ ID NO: 149 - DNA, 20 bp, synthetic construct
  source 1..20: mol_type = other DNA
ccttctactattaggaagtt

SEQ ID NO: 150 - DNA, 20 bp, synthetic construct
  source 1..20: mol_type = other DNA
caagaatccttctactatta

SEQ ID NO: 151 - DNA, 20 bp, synthetic construct
  source 1..20: mol_type = other DNA
tctccccaagaatccttcta

SEQ ID NO: 152 - DNA, 20 bp, synthetic construct
  source 1..20: mol_type = other DNA
agacatactcttctccttca

SEQ ID NO: 153 - DNA, 20 bp, synthetic construct
  source 1..20: mol_type = other DNA
acaggttctagacatactct

SEQ ID NO: 154 - DNA, 20 bp, synthetic construct
  source 1..20: mol_type = other DNA
ttgcattttctacaggttct

SEQ ID NO: 155 - DNA, 20 bp, synthetic construct
  source 1..20: mol_type = other DNA
ggctctgcttgcattttcta

SEQ ID NO: 156 - DNA, 20 bp, synthetic construct
  source 1..20: mol_type = other DNA
cagcttaaatcctagaccag

SEQ ID NO: 157 - DNA, 20 bp, synthetic construct
  source 1..20: mol_type = other DNA
gtacctgcagcttaaatcct

SEQ ID NO: 158 - DNA, 20 bp, synthetic construct
  source 1..20: mol_type = other DNA
tatccattagactaggcagg

SEQ ID NO: 159 - DNA, 20 bp, synthetic construct
  source 1..20: mol_type = other DNA
tcaacaacaatatccattag

SEQ ID NO: 160 - DNA, 20 bp, synthetic construct
  source 1..20: mol_type = other DNA
aacaataccatcaacaacaa

SEQ ID NO: 161 - DNA, 20 bp, synthetic construct
  source 1..20: mol_type = other DNA
actgacggatctggtttcaa

SEQ ID NO: 162 - DNA, 20 bp, synthetic construct
  source 1..20: mol_type = other DNA
atgcaccagagactcgaatc

SEQ ID NO: 163 - DNA, 20 bp, synthetic construct
  source 1..20: mol_type = other DNA
tgtaaagttcctttccgcct

SEQ ID NO: 164 - DNA, 20 bp, synthetic construct
  source 1..20: mol_type = other DNA
acacatctttaagatgagcg

SEQ ID NO: 165 - DNA, 20 bp, synthetic construct
  source 1..20: mol_type = other DNA
tgaccttgggcaagaacatt

SEQ ID NO: 166 - DNA, 20 bp, synthetic construct
  source 1..20: mol_type = other DNA
agttggcctgaaaggcaaaa

SEQ ID NO: 167 - DNA, 20 bp, synthetic construct
  source 1..20: mol_type = other DNA
ttcttcgaatcactcagcca

SEQ ID NO: 168 - DNA, 20 bp, synthetic construct
  source 1..20: mol_type = other DNA
ttcctcactttcttcgaatc

SEQ ID NO: 169 - DNA, 20 bp, synthetic construct
  source 1..20: mol_type = other DNA
agggaggattcctcactttc

SEQ ID NO: 170 - DNA, 20 bp, synthetic construct
  source 1..20: mol_type = other DNA
attgactgaaagacgacgaa

SEQ ID NO: 171 - DNA, 20 bp, synthetic construct
  source 1..20: mol_type = other DNA
agagtggaagagattgactg

SEQ ID NO: 172 - DNA, 20 bp, synthetic construct
  source 1..20: mol_type = other DNA
tcaatccttagagtggaaga

SEQ ID NO: 173 - DNA, 20 bp, synthetic construct
  source 1..20: mol_type = other DNA
cgctcactcaatccttagag

SEQ ID NO: 174 - DNA, 20 bp, synthetic construct
  source 1..20: mol_type = other DNA
cagcaagcacctttgagaga

SEQ ID NO: 175 - DNA, 20 bp, synthetic construct
  source 1..20: mol_type = other DNA
tgttctgatagcctggtgga

SEQ ID NO: 176 - DNA, 20 bp, synthetic construct
  source 1..20: mol_type = other DNA
tgtttaagccaccccctgtt

SEQ ID NO: 177 - DNA, 20 bp, synthetic construct
  source 1..20: mol_type = other DNA
ttccatgctgtttaagccac

SEQ ID NO: 178 - DNA, 20 bp, synthetic construct
  source 1..20: mol_type = other DNA
tgagattccatgctgtttaa

SEQ ID NO: 179 - DNA, 20 bp, synthetic construct
  source 1..20: mol_type = other DNA
gagaacggaaagctgagatt

SEQ ID NO: 180 - DNA, 20 bp, synthetic construct
  source 1..20: mol_type = other DNA
ttcctctggagaacggaaag

SEQ ID NO: 181 - DNA, 20 bp, synthetic construct
  source 1..20: mol_type = other DNA
cctctaatcctcagcatttt

SEQ ID NO: 182 - DNA, 20 bp, synthetic construct
  source 1..20: mol_type = other DNA
tcctatccctgcctctaatc

SEQ ID NO: 183 - DNA, 20 bp, synthetic construct
  source 1..20: mol_type = other DNA
ttggttctctccaggtccta

SEQ ID NO: 184 - DNA, 20 bp, synthetic construct
  source 1..20: mol_type = other DNA
cattacagtaccttggttct

SEQ ID NO: 185 - DNA, 20 bp, synthetic construct
  source 1..20: mol_type = other DNA
agaacatcattacagtacct

SEQ ID NO: 186 - DNA, 20 bp, synthetic construct
  source 1..20: mol_type = other DNA
ttctggataaagaacatcat

SEQ ID NO: 187 - DNA, 20 bp, synthetic construct
  source 1..20: mol_type = other DNA
ggctgtattctggataaaga

SEQ ID NO: 188 - DNA, 20 bp, synthetic construct
  source 1..20: mol_type = other DNA
tgctggcatcttcaaggaaa

SEQ ID NO: 189 - DNA, 20 bp, synthetic construct
  source 1..20: mol_type = other DNA
attacaaaccttcccagcct

SEQ ID NO: 190 - DNA, 20 bp, synthetic construct
  source 1..20: mol_type = other DNA
ttgggtcaccgtattacaaa

SEQ ID NO: 191 - DNA, 20 bp, synthetic construct
  source 1..20: mol_type = other DNA
gtgtcttgggtcaccgtatt

SEQ ID NO: 192 - DNA, 20 bp, synthetic construct
  source 1..20: mol_type = other DNA
tccaaatcttcctctctcct

SEQ ID NO: 193 - DNA, 20 bp, synthetic construct
  source 1..20: mol_type = other DNA
aaggagggagtctttgctgt

SEQ ID NO: 194 - DNA, 20 bp, synthetic construct
  source 1..20: mol_type = other DNA
gaacaaattcttcatccatc

SEQ ID NO: 195 - DNA, 20 bp, synthetic construct
  source 1..20: mol_type = other DNA
gataagggaacaaattcttc

SEQ ID NO: 196 - DNA, 20 bp, synthetic construct
  source 1..20: mol_type = other DNA
gtctgtccatctgagataag

SEQ ID NO: 197 - DNA, 20 bp, synthetic construct
  source 1..20: mol_type = other DNA
aaacaacatgctcaggatca

SEQ ID NO: 198 - DNA, 20 bp, synthetic construct
  source 1..20: mol_type = other DNA
tcttagagcagaggctcaga

SEQ ID NO: 199 - DNA, 20 bp, synthetic construct
  source 1..20: mol_type = other DNA
ttattcccatcttagagcag

SEQ ID NO: 200 - DNA, 20 bp, synthetic construct
  source 1..20: mol_type = other DNA
tcatgccaatcctatagagt

SEQ ID NO: 201 - DNA, 20 bp, synthetic construct
  source 1..20: mol_type = other DNA
tcatttagtcctcatgccaa

SEQ ID NO: 202 - DNA, 20 bp, synthetic construct
  source 1..20: mol_type = other DNA
atagacactttagatgcatt

SEQ ID NO: 203 - DNA, 20 bp, synthetic construct
  source 1..20: mol_type = other DNA
tcttctcactaatagacact

SEQ ID NO: 204 - DNA, 20 bp, synthetic construct
  source 1..20: mol_type = other DNA
gtatggagtatcttctcact

SEQ ID NO: 205 - DNA, 20 bp, synthetic construct
  source 1..20: mol_type = other DNA
ccactgtgtatggagtatct

SEQ ID NO: 206 - DNA, 20 bp, synthetic construct
  source 1..20: mol_type = other DNA
aaaacaagccactgtgtatg

SEQ ID NO: 207 - DNA, 20 bp, synthetic construct
  source 1..20: mol_type = other DNA
ttatgatcaaaacaagccac

SEQ ID NO: 208 - DNA, 20 bp, synthetic construct
  source 1..20: mol_type = other DNA
gggaaccatttatgatcaaa

SEQ ID NO: 209 - DNA, 20 bp, synthetic construct
  source 1..20: mol_type = other DNA
ggaaataaatagggaaccat

SEQ ID NO: 210 - DNA, 20 bp, synthetic construct
  source 1..20: mol_type = other DNA
tgggctgccctggaaataaa

SEQ ID NO: 211 - DNA, 20 bp, synthetic construct
  source 1..20: mol_type = other DNA
taatattgggctgccctgga

SEQ ID NO: 212 - DNA, 20 bp, synthetic construct
  source 1..20: mol_type = other DNA
taggaacctgtaatattggg

SEQ ID NO: 213 - DNA, 20 bp, synthetic construct
  source 1..20: mol_type = other DNA
gaaaggagtaggaacctgta

SEQ ID NO: 214 - DNA, 20 bp, synthetic construct
  source 1..20: mol_type = other DNA
ttcattctcttgaaaggagt

SEQ ID NO: 215 - DNA, 20 bp, synthetic construct
  source 1..20: mol_type = other DNA
tgacttcctaatacaaagaa

SEQ ID NO: 216 - DNA, 20 bp, synthetic construct
  source 1..20: mol_type = other DNA
caacagtcttgacttcctaa

SEQ ID NO: 217 - DNA, 20 bp, synthetic construct
  source 1..20: mol_type = other DNA
aagttgccaacagtcttgac

SEQ ID NO: 218 - DNA, 20 bp, synthetic construct
  source 1..20: mol_type = other DNA
tttcaaccgccttgactttc

SEQ ID NO: 219 - DNA, 20 bp, synthetic construct
  source 1..20: mol_type = other DNA
gatctggtttcaaccgcctt

SEQ ID NO: 220 - DNA, 20 bp, synthetic construct
  source 1..20: mol_type = other DNA
ttcaacgacgcctttgtcta

SEQ ID NO: 221 - DNA, 20 bp, synthetic construct
  source 1..20: mol_type = other DNA
agagactcgaatcccagcta

SEQ ID NO: 222 - DNA, 20 bp, synthetic construct
  source 1..20: mol_type = other DNA
gggcattttcctaaatctgt

SEQ ID NO: 223 - DNA, 20 bp, synthetic construct
  source 1..20: mol_type = other DNA
gatgctcccttacacatctt

SEQ ID NO: 224 - DNA, 20 bp, synthetic construct
  source 1..20: mol_type = other DNA
ttctcaccgatgctccctta

SEQ ID NO: 225 - DNA, 20 bp, synthetic construct
  source 1..20: mol_type = other DNA
tgaaccctcactatgactcc

SEQ ID NO: 226 - DNA, 20 bp, synthetic construct
  source 1..20: mol_type = other DNA
aactaggattcaaacctcca

SEQ ID NO: 227 - DNA, 20 bp, synthetic construct
  source 1..20: mol_type = other DNA
caatcctatagagtttggaa

SEQ ID NO: 228 - DNA, 20 bp, synthetic construct
  source 1..20: mol_type = other DNA
gaactgggtgattagctgta

SEQ ID NO: 229 - DNA, 20 bp, synthetic construct
  source 1..20: mol_type = other DNA
cattcatcaactgaggtaca

SEQ ID NO: 230 - DNA, 20 bp, synthetic construct
  source 1..20: mol_type = other DNA
cacttcccaggttagataga

SEQ ID NO: 231 - DNA, 20 bp, synthetic construct
  source 1..20: mol_type = other DNA
acacaatcacactccacttc

SEQ ID NO: 232 - DNA, 20 bp, synthetic construct
  source 1..20: mol_type = other DNA
acacgtccttccactaacaa

SEQ ID NO: 233 - DNA, 20 bp, synthetic construct
  source 1..20: mol_type = other DNA
attcatccatgcagagagaa

SEQ ID NO: 234 - DNA, 20 bp, synthetic construct
  source 1..20: mol_type = other DNA
ttgcagtctctcagcaccat

SEQ ID NO: 235 - DNA, 20 bp, synthetic construct
  source 1..20: mol_type = other DNA
aatcttcactcatacccaca

SEQ ID NO: 236 - DNA, 20 bp, synthetic construct
  source 1..20: mol_type = other DNA
cacacttataatcttcactc

SEQ ID NO: 237 - DNA, 20 bp, synthetic construct
  source 1..20: mol_type = other DNA
acttaaagtgtaaagtacag

SEQ ID NO: 238 - DNA, 20 bp, synthetic construct
  source 1..20: mol_type = other DNA
tgctgccacttaaagtgtaa

SEQ ID NO: 239 - DNA, 20 bp, synthetic construct
  source 1..20: mol_type = other DNA
taagcactatgctgccactt

SEQ ID NO: 240 - DNA, 20 bp, synthetic construct
  source 1..20: mol_type = other DNA
ctgccatggttaagcactat

SEQ ID NO: 241 - DNA, 20 bp, synthetic construct
  source 1..20: mol_type = other DNA
caataatcctaaaagaaggg

SEQ ID NO: 242 - DNA, 20 bp, synthetic construct
  source 1..20: mol_type = other DNA
ttaactcttctaattctcac

SEQ ID NO: 243 - DNA, 20 bp, synthetic construct
  source 1..20: mol_type = other DNA
tcaagcccctaacatatatt

SEQ ID NO: 244 - DNA, 20 bp, synthetic construct
  source 1..20: mol_type = other DNA
tacatgccaggtatcaagcc

SEQ ID NO: 245 - DNA, 20 bp, synthetic construct
  source 1..20: mol_type = other DNA
gaacacttaattagctctta

SEQ ID NO: 246 - DNA, 20 bp, synthetic construct
  source 1..20: mol_type = other DNA
tactctgtagttatgagaaa

SEQ ID NO: 247 - DNA, 20 bp, synthetic construct
  source 1..20: mol_type = other DNA
caaactactctgtagttatg

SEQ ID NO: 248 - DNA, 20 bp, synthetic construct
  source 1..20: mol_type = other DNA
aatatcaaactactctgtag

SEQ ID NO: 249 - DNA, 20 bp, synthetic construct
  source 1..20: mol_type = other DNA
tccctgaaatatcaaactac

SEQ ID NO: 250 - DNA, 20 bp, synthetic construct
  source 1..20: mol_type = other DNA
agcagtgggaaacaaacata

SEQ ID NO: 251 - DNA, 20 bp, synthetic construct
  source 1..20: mol_type = other DNA
tacaacatagggttgttgtg

SEQ ID NO: 252 - DNA, 20 bp, synthetic construct
  source 1..20: mol_type = other DNA
agtgctaattacaacatagg

SEQ ID NO: 253 - DNA, 20 bp, synthetic construct
  source 1..20: mol_type = other DNA
gccagtggaacagtgctaat

SEQ ID NO: 254 - DNA, 20 bp, synthetic construct
  source 1..20: mol_type = other DNA
gtctttaggtgccagtggaa

SEQ ID NO: 255 - DNA, 20 bp, synthetic construct
  source 1..20: mol_type = other DNA
ttaacttgtacctgcagcat

SEQ ID NO: 256 - DNA, 20 bp, synthetic construct
  source 1..20: mol_type = other DNA
gagattaacttgtacctgca

SEQ ID NO: 257 - DNA, 16 bp, synthetic construct
  source 1..16: mol_type = other DNA
attgcggcagcatttc

SEQ ID NO: 258 - DNA, 16 bp, synthetic construct
  source 1..16: mol_type = other DNA
gaatacagagtcccga

SEQ ID NO: 259 - DNA, 16 bp, synthetic construct
  source 1..16: mol_type = other DNA
gttactttattggttg

SEQ ID NO: 260 - DNA, 20 bp, synthetic construct
  source 1..20: mol_type = other DNA
aatgttgttaagttgccaac

SEQ ID NO: 261 - DNA, 20 bp, synthetic construct
  source 1..20: mol_type = other DNA
aaggaaatgtggcacgtcta

SEQ ID NO: 262 - DNA, 20 bp, synthetic construct
  source 1..20: mol_type = other DNA
atgcccaagacacatgcaca

SEQ ID NO: 263 - DNA, 20 bp, synthetic construct
  source 1..20: mol_type = other DNA
caacgcaaatgcccaagaca

SEQ ID NO: 264 - DNA, 20 bp, synthetic construct
  source 1..20: mol_type = other DNA
gttagaatggagatccttaa

SEQ ID NO: 265 - DNA, 20 bp, synthetic construct
  source 1..20: mol_type = other DNA
tagaacgtgggcgaaggata

SEQ ID NO: 266 - DNA, 20 bp, synthetic construct
  source 1..20: mol_type = other DNA
gatccaattaaactacagag

SEQ ID NO: 267 - DNA, 20 bp, synthetic construct
  source 1..20: mol_type = other DNA
ggaagcatcacgctaactga

SEQ ID NO: 268 - DNA, 20 bp, synthetic construct
  source 1..20: mol_type = other DNA
taagaaactgcagtaaagtc

SEQ ID NO: 269 - DNA, 20 bp, synthetic construct
  source 1..20: mol_type = other DNA
taagctgataagaaactgca

SEQ ID NO: 270 - DNA, 20 bp, synthetic construct
  source 1..20: mol_type = other DNA
acaaagaggagttgctggta

SEQ ID NO: 271 - DNA, 20 bp, synthetic construct
  source 1..20: mol_type = other DNA
aacactaattagcaaatgca

SEQ ID NO: 272 - DNA, 20 bp, synthetic construct
  source 1..20: mol_type = other DNA
aaagatatccaagacttgaa

SEQ ID NO: 273 - DNA, 20 bp, synthetic construct
  source 1..20: mol_type = other DNA
gaaactttaacccccactgt

SEQ ID NO: 274 - DNA, 20 bp, synthetic construct
  source 1..20: mol_type = other DNA
agactccgacataataatag

SEQ ID NO: 275 - DNA, 20 bp, synthetic construct
  source 1..20: mol_type = other DNA
acaactggaatcagcaactg

SEQ ID NO: 276 - DNA, 20 bp, synthetic construct
  source 1..20: mol_type = other DNA
aaggaacaactggaatcagc

SEQ ID NO: 277 - DNA, 20 bp, synthetic construct
  source 1..20: mol_type = other DNA
ttttctcatcaacaggcctg

SEQ ID NO: 278 - DNA, 20 bp, synthetic construct
  source 1..20: mol_type = other DNA
cccttcagactaactgcaga

SEQ ID NO: 279 - DNA, 20 bp, synthetic construct
  source 1..20: mol_type = other DNA
aaggttgggttacccactat

SEQ ID NO: 280 - DNA, 20 bp, synthetic construct
  source 1..20: mol_type = other DNA
tgaagcctatacaagtatca

SEQ ID NO: 281 - DNA, 20 bp, synthetic construct
  source 1..20: mol_type = other DNA
gagaacgtcatgaagcctat

SEQ ID NO: 282 - DNA, 20 bp, synthetic construct
  source 1..20: mol_type = other DNA
aagaaaggtaagaaccttga

SEQ ID NO: 283 - DNA, 20 bp, synthetic construct
  source 1..20: mol_type = other DNA
ctaaccccaatgcaagaaag

SEQ ID NO: 284 - DNA, 20 bp, synthetic construct
  source 1..20: mol_type = other DNA
agcatgttctaaccccaatg

SEQ ID NO: 285 - DNA, 20 bp, synthetic construct
  source 1..20: mol_type = other DNA
atttccgtgtctcctgactg

SEQ ID NO: 286 - DNA, 20 bp, synthetic construct
  source 1..20: mol_type = other DNA
agtccctgatttccgtgtct

SEQ ID NO: 287 - DNA, 20 bp, synthetic construct
  source 1..20: mol_type = other DNA
aactctcaagcttggtaggg

SEQ ID NO: 288 - DNA, 20 bp, synthetic construct
  source 1..20: mol_type = other DNA
agttgacctggaactctcaa

SEQ ID NO: 289 - DNA, 20 bp, synthetic construct
  source 1..20: mol_type = other DNA
tctggagcagatactacact

SEQ ID NO: 290 - DNA, 20 bp, synthetic construct
  source 1..20: mol_type = other DNA
aatagtgcactctggagcag

SEQ ID NO: 291 - DNA, 20 bp, synthetic construct
  source 1..20: mol_type = other DNA
actgtgccgtgaggaatagt

SEQ ID NO: 292 - DNA, 20 bp, synthetic construct
  source 1..20: mol_type = other DNA
attttcaaatgaggtacgtg

SEQ ID NO: 293 - DNA, 20 bp, synthetic construct
  source 1..20: mol_type = other DNA
tcccagtgaatcaatgcaga

SEQ ID NO: 294 - DNA, 20 bp, synthetic construct
  source 1..20: mol_type = other DNA
gatttaggttcagctttcaa

SEQ ID NO: 295 - DNA, 20 bp, synthetic construct
  source 1..20: mol_type = other DNA
aaggaaagtggctgacagat

SEQ ID NO: 296 - DNA, 20 bp, synthetic construct
  source 1..20: mol_type = other DNA
tgattagctgtagaggacaa

SEQ ID NO: 297 - DNA, 20 bp, synthetic construct
  source 1..20: mol_type = other DNA
caaatggaatcacaggacct

SEQ ID NO: 298 - DNA, 20 bp, synthetic construct
  source 1..20: mol_type = other DNA
cctgctcccaaatggaatca

SEQ ID NO: 299 - DNA, 20 bp, synthetic construct
  source 1..20: mol_type = other DNA
aagatcacctgcaaatccct

SEQ ID NO: 300 - DNA, 20 bp, synthetic construct
  source 1..20: mol_type = other DNA
tgggcttcacatacagcaga

SEQ ID NO: 301 - DNA, 20 bp, synthetic construct
  source 1..20: mol_type = other DNA
gatacagggagattaacttg

SEQ ID NO: 302 - DNA, 20 bp, synthetic construct
  source 1..20: mol_type = other DNA
agtaagggtaagtgggcaga

SEQ ID NO: 303 - DNA, 20 bp, synthetic construct
  source 1..20: mol_type = other DNA
atcaatgcactttctctttc

SEQ ID NO: 304 - DNA, 20 bp, synthetic construct
  source 1..20: mol_type = other DNA
ccatcaatgcactttctctt

SEQ ID NO: 305 - DNA, 20 bp, synthetic construct
  source 1..20: mol_type = other DNA
cctggccatcaatgcacttt

SEQ ID NO: 306 - DNA, 20 bp, synthetic construct
  source 1..20: mol_type = other DNA
ttagaacaggctgagggtca

SEQ ID NO: 307 - DNA, 20 bp, synthetic construct
  source 1..20: mol_type = other DNA
tcttttagaacaggctgagg

SEQ ID NO: 308 - DNA, 20 bp, synthetic construct
  source 1..20: mol_type = other DNA
ctcttcttttagaacaggct

SEQ ID NO: 309 - DNA, 20 bp, synthetic construct
  source 1..20: mol_type = other DNA
attataggcatgagccacca

SEQ ID NO: 310 - DNA, 20 bp, synthetic construct
  source 1..20: mol_type = other DNA
ttggtcaggctggtcttgaa

SEQ ID NO: 311 - DNA, 20 bp, synthetic construct
  source 1..20: mol_type = other DNA
gggtttctccatgttggtca

SEQ ID NO: 312 - DNA, 20 bp, synthetic construct
  source 1..20: mol_type = other DNA
ccaccacacccattaaattt

SEQ ID NO: 313 - DNA, 20 bp, synthetic construct
  source 1..20: mol_type = other DNA
aagcaattctcctgcctcag

SEQ ID NO: 314 - DNA, 20 bp, synthetic construct
  source 1..20: mol_type = other DNA
tgtctcccaggttcaagcaa

SEQ ID NO: 315 - DNA, 20 bp, synthetic construct
  source 1..20: mol_type = other DNA
atctcagctcaccacaacct

SEQ ID NO: 316 - DNA, 20 bp, synthetic construct
  source 1..20: mol_type = other DNA
agtgcaatggcgtgatctca

SEQ ID NO: 317 - DNA, 20 bp, synthetic construct
  source 1..20: mol_type = other DNA
agtttcgctcttgttgccca

SEQ ID NO: 318 - DNA, 20 bp, synthetic construct
  source 1..20: mol_type = other DNA
tgtttttaatttgagatgga

SEQ ID NO: 319 - DNA, 20 bp, synthetic construct
  source 1..20: mol_type = other DNA
caccaagctgttttttgttt

SEQ ID NO: 320 - DNA, 20 bp, synthetic construct
  source 1..20: mol_type = other DNA
ggtaccaccaagctgttttt

SEQ ID NO: 321 - DNA, 20 bp, synthetic construct
  source 1..20: mol_type = other DNA
atttcaacccaagggtacca

SEQ ID NO: 322 - DNA, 20 bp, synthetic construct
  source 1..20: mol_type = other DNA
accacgagatttcaacccaa

SEQ ID NO: 323 - DNA, 20 bp, synthetic construct
  source 1..20: mol_type = other DNA
acatgacaaccacgagattt

SEQ ID NO: 324 - DNA, 20 bp, synthetic construct
  source 1..20: mol_type = other DNA
cactattggattctatcagt

SEQ ID NO: 325 - DNA, 20 bp, synthetic construct
  source 1..20: mol_type = other DNA
tctgcactattggattctat

SEQ ID NO: 326 - DNA, 20 bp, synthetic construct
  source 1..20: mol_type = other DNA
agatttcaattgctcatctc

SEQ ID NO: 327 - DNA, 20 bp, synthetic construct
  source 1..20: mol_type = other DNA
tctagatttcaattgctcat

SEQ ID NO: 328 - DNA, 20 bp, synthetic construct
  source 1..20: mol_type = other DNA
agataactgtgactcaggga

SEQ ID NO: 329 - DNA, 20 bp, synthetic construct
  source 1..20: mol_type = other DNA
taagcgagataactgtgact

SEQ ID NO: 330 - DNA, 20 bp, synthetic construct
  source 1..20: mol_type = other DNA
gcattttctacaggttctag

SEQ ID NO: 331 - DNA, 20 bp, synthetic construct
  source 1..20: mol_type = other DNA
gcttgcattttctacaggtt

SEQ ID NO: 332 - DNA, 20 bp, synthetic construct
  source 1..20: mol_type = other DNA
tctgcttgcattttctacag

SEQ ID NO: 333 - DNA, 20 bp, synthetic construct
  source 1..20: mol_type = other DNA
acctgcagcttaaatcctag

SEQ ID NO: 334 - DNA, 20 bp, synthetic construct
  source 1..20: mol_type = other DNA
gagtacctgcagcttaaatc

SEQ ID NO: 335 - DNA, 20 bp, synthetic construct
  source 1..20: mol_type = other DNA
aggagtacctgcagcttaaa

SEQ ID NO: 336 - DNA, 20 bp, synthetic construct
  source 1..20: mol_type = other DNA
gaaggtatctcaaagtaaca

SEQ ID NO: 337 - DNA, 20 bp, synthetic construct
  source 1..20: mol_type = other DNA
agagcctcctccctaattca

SEQ ID NO: 338 - DNA, 20 bp, synthetic construct
  source 1..20: mol_type = other DNA
cacaagctgggtttttgaaa

SEQ ID NO: 339 - DNA, 20 bp, synthetic construct
  source 1..20: mol_type = other DNA
gcataaccttacatggaaac

SEQ ID NO: 340 - DNA, 20 bp, synthetic construct
  source 1..20: mol_type = other DNA
tcaagaccgcataaccttac

SEQ ID NO: 341 - DNA, 20 bp, synthetic construct
  source 1..20: mol_type = other DNA
aaaacacaggcacagaactg

SEQ ID NO: 342 - DNA, 20 bp, synthetic construct
  source 1..20: mol_type = other DNA
ttgtgtgtaaaacacaggca

SEQ ID NO: 343 - DNA, 20 bp, synthetic construct
  source 1..20: mol_type = other DNA
tcatggttgcttccaacttt

SEQ ID NO: 344 - DNA, 20 bp, synthetic construct
  source 1..20: mol_type = other DNA
gccaaatccattcatcaact

SEQ ID NO: 345 - DNA, 20 bp, synthetic construct
  source 1..20: mol_type = other DNA
agagaaaccacacgtccttc

SEQ ID NO: 346 - DNA, 20 bp, synthetic construct
  source 1..20: mol_type = other DNA
catgaccctccaaatacact

SEQ ID NO: 347 - DNA, 20 bp, synthetic construct
  source 1..20: mol_type = other DNA
ctgcagagtctatgtgttaa

SEQ ID NO: 348 - DNA, 20 bp, synthetic construct
  source 1..20: mol_type = other DNA
aatctagctgcagagtctat

SEQ ID NO: 349 - DNA, 20 bp, synthetic construct
  source 1..20: mol_type = other DNA
ttgaaccccaagaaatctag

SEQ ID NO: 350 - DNA, 20 bp, synthetic construct
  source 1..20: mol_type = other DNA
gttgtgaaagcagtgggaaa

SEQ ID NO: 351 - DNA, 20 bp, synthetic construct
  source 1..20: mol_type = other DNA
tcagaaattgggagtgacac

SEQ ID NO: 352 - DNA, 20 bp, synthetic construct
  source 1..20: mol_type = other DNA
gtggctggagctcagaaatt

SEQ ID NO: 353 - DNA, 20 bp, synthetic construct
  source 1..20: mol_type = other DNA
aactttctctcctcactgct

SEQ ID NO: 354 - DNA, 20 bp, synthetic construct
  source 1..20: mol_type = other DNA
cctgaaaggcaaaagctgaa

SEQ ID NO: 355 - DNA, 20 bp, synthetic construct
  source 1..20: mol_type = other DNA
aatttcaggttaatatccct

SEQ ID NO: 356 - DNA, 20 bp, synthetic construct
  source 1..20: mol_type = other DNA
gtctgactgctagccatact

SEQ ID NO: 357 - DNA, 20 bp, synthetic construct
  source 1..20: mol_type = other DNA
aacatcaacaaaatagtctg

SEQ ID NO: 358 - DNA, 20 bp, synthetic construct
  source 1..20: mol_type = other DNA
aatgaattcacaagctgggt

SEQ ID NO: 359 - DNA, 20 bp, synthetic construct
  source 1..20: mol_type = other DNA
gatcagagagaactaaagga

SEQ ID NO: 360 - DNA, 20 bp, synthetic construct
  source 1..20: mol_type = other DNA
actcactcaagaccgcataa

SEQ ID NO: 361 - DNA, 20 bp, synthetic construct
  source 1..20: mol_type = other DNA
aaggcccatccaaagatcat

SEQ ID NO: 362 - DNA, 20 bp, synthetic construct
  source 1..20: mol_type = other DNA
tcaagtgagtccctgatttc

SEQ ID NO: 363 - DNA, 20 bp, synthetic construct
  source 1..20: mol_type = other DNA
caagagattcctttgggtgc

SEQ ID NO: 364 - DNA, 20 bp, synthetic construct
  source 1..20: mol_type = other DNA
agtagggtagggcatcatct

SEQ ID NO: 365 - DNA, 20 bp, synthetic construct
  source 1..20: mol_type = other DNA
aaatgaggtacgtggctcat

SEQ ID NO: 366 - DNA, 20 bp, synthetic construct
  source 1..20: mol_type = other DNA
aggttcagctttcaagatgg

SEQ ID NO: 367 - DNA, 20 bp, synthetic construct
  source 1..20: mol_type = other DNA
tgtagaggacaaggaaagtg

SEQ ID NO: 368 - DNA, 20 bp, synthetic construct
  source 1..20: mol_type = other DNA
gaggtacatcatggttgctt

SEQ ID NO: 369 - DNA, 20 bp, synthetic construct
  source 1..20: mol_type = other DNA
agagaaaccacacgtccttc

SEQ ID NO: 370 - DNA, 20 bp, synthetic construct
  source 1..20: mol_type = other DNA
tccaaatacactcattcatc

SEQ ID NO: 371 - DNA, 20 bp, synthetic construct
  source 1..20: mol_type = other DNA
cagaattgaggcagaatttg

SEQ ID NO: 372 - DNA, 20 bp, synthetic construct
  source 1..20: mol_type = other DNA
aaggtcacacagaattgagg

SEQ ID NO: 373 - DNA, 20 bp, synthetic construct
  source 1..20: mol_type = other DNA
ctgttaatatttccttgtgt

SEQ ID NO: 374 - DNA, 20 bp, synthetic construct
  source 1..20: mol_type = other DNA
gagggatctgttaatatttc

SEQ ID NO: 375 - DNA, 20 bp, synthetic construct
  source 1..20: mol_type = other DNA
aaattgggagtgacacagga

SEQ ID NO: 376 - DNA, 20 bp, synthetic construct
  source 1..20: mol_type = other DNA
agaaactttctctcctcact

SEQ ID NO: 377 - DNA, 20 bp, synthetic construct
  source 1..20: mol_type = other DNA
gcagaaactttctctcctca

SEQ ID NO: 378 - DNA, 20 bp, synthetic construct
  source 1..20: mol_type = other DNA
atacagagtcccgaaaaagg

SEQ ID NO: 379 - DNA, 20 bp, synthetic construct
  source 1..20: mol_type = other DNA
ggaatacagagtcccgaaaa

SEQ ID NO: 380 - DNA, 20 bp, synthetic construct
  source 1..20: mol_type = other DNA
ggttactttattggttggga

SEQ ID NO: 381 - DNA, 20 bp, synthetic construct
  source 1..20: mol_type = other DNA
tggttactttattggttggg

SEQ ID NO: 382 - DNA, 20 bp, synthetic construct
  source 1..20: mol_type = other DNA
agtggttactttattggttg

SEQ ID NO: 383 - DNA, 20 bp, synthetic construct
  source 1..20: mol_type = other DNA
tcccaaattgcagccatcag

SEQ ID NO: 384 - DNA, 20 bp, synthetic construct
  source 1..20: mol_type = other DNA
ttcagcacagaatcctccca

SEQ ID NO: 385 - DNA, 20 bp, synthetic construct
  source 1..20: mol_type = other DNA
aattctcagtctctggccct

SEQ ID NO: 386 - DNA, 20 bp, synthetic construct
  source 1..20: mol_type = other DNA
aaggaattctcagtctctgg